European Patent Application EP 4 763 984 A1, published June 24, 2026. Title: RNA PRODUCTS AND METHODS OF PRODUCTION. Applicant: 4basebio UK Ltd. The sequence listing filed with the application follows.

SEQUENCE LISTING (8 sequences)

SEQ ID NO: 1 - RNA, 20 nt, synthetic construct
  source 1..20: mol_type = other RNA
  modified_base 2..4: mod_base = OTHER; note = phosphorothioated nucleotide
ctcgtgaccaccctgagcca

SEQ ID NO: 2 - RNA, 108 nt, synthetic construct
  source 1..108: mol_type = other RNA
ggttttagagctagaaatagcaagttaaaataaggctagtccgttatcaacttgaaaaagtggcaccgagtcggtgcggtagcgggcgaagcactgcacgccgtaggt

SEQ ID NO: 3 - RNA, 16 nt, synthetic construct
  source 1..16: mol_type = other RNA
  modified_base 14..16: mod_base = OTHER; note = phosphorothioated nucleotide
gaaggtggtcacgagg

SEQ ID NO: 4 - DNA, 144 bp, synthetic construct
  source 1..144: mol_type = other DNA
cctcgtgaccaccttcacctacggcgtgcagtgcttcgcccgctaccgcaccgactcggtgccactttttcaagttgataacggactagccttattttaacttgctatttctagctctaaaacctggctcagggtggtcacgag

SEQ ID NO: 5 - DNA, 133 bp, synthetic construct
  source 1..133: mol_type = other DNA
ccctcgagtaatacgactcactataggttttagagctagaaatagcaagttaaaataaggctagtccgttatcaacttgaaaaagtggcaccgagtcggtgcggtagcgggcgaagcactgcacgccgtaggt

SEQ ID NO: 6 - RNA, 144 nt, synthetic construct
  source 1..144: mol_type = other RNA
  modified_base 2..4: mod_base = OTHER; note = phosphorothioated nucleotide
  modified_base 142..144: mod_base = OTHER; note = phosphorothioated nucleotide
ctcgtgaccaccctgagccaggttttagagctagaaatagcaagttaaaataaggctagtccgttatcaacttgaaaaagtggcaccgagtcggtgcggtagcgggcgaagcactgcacgccgtaggtgaaggtggtcacgagg

SEQ ID NO: 7 - DNA, 171 bp, synthetic construct
  source 1..171: mol_type = other DNA
ccctcgagtaatacgactcactataggctcgtgaccaccctgagccaggttttagagctagaaatagcaagttaaaataaggctagtccgttatcaacttgaaaaagtggcaccgagtcggtgcggtagcgggcgaagcactgcacgccgtaggtgaaggtggtcacgagg

SEQ ID NO: 8 - RNA, 146 nt, synthetic construct
  source 1..146: mol_type = other RNA
ggctcgtgaccaccctgagccaggttttagagctagaaatagcaagttaaaataaggctagtccgttatcaacttgaaaaagtggcaccgagtcggtgcggtagcgggcgaagcactgcacgccgtaggtgaaggtggtcacgagg